European Patent Application EP 4 368 708 A1, published May 15, 2024. Title: Nucleic Acid Ligase. Applicant: WENZHOU MEDICAL UNIVERSITY. The sequence listing filed with the application follows.

SEQUENCE LISTING (7 sequences)

SEQ ID NO: 1 - protein, 390 aa, artificial sequence
  HyperLigase
MTWIKNPEPWMVNLVAEKLGLDVERVETLARHGTIRFRGYRDVVYALLRREIAGHPEGTVVLLERNGARLVPGYPPIQRMVLPTIALPRHFIDKVVVEEAMNGYNVRLVMFHRKLLAVTRGGFICPYTTARLERLIGGRVRELFREIDPETYTIAGEVVGLENPYTRYFYPEAPRFDYFVFDLFHELKPLPPLERNELLEKYGLKHVRLLGVIDKNDVEMFKQIVAELDREGREGVVAKDPEYRVPPLKYTTSAVNIGDVRYGMRFFMEEGRSFLFSRLLRELFRAYEEGFGDAQLEKLALEFGRAATEPALESIRKVAMGDMLYEEFELVFADEVELEEFTSYMAELGVDIVVVSTSREDEGLRARMRKIKDTWIQLRKVLDTGLSPVD

SEQ ID NO: 2 - protein, 390 aa, artificial sequence
  R79 mutant of Hyperligase
  misc_feature (79)..(79): Xaa can be any amino acid except Arg
MTWIKNPEPWMVNLVAEKLGLDVERVETLARHGTIRFRGYRDVVYALLRREIAGHPEGTVVLLERNGARLVPGYPPIQXMVLPTIALPRHFIDKVVVEEAMNGYNVRLVMFHRKLLAVTRGGFICPYTTARLERLIGGRVRELFREIDPETYTIAGEVVGLENPYTRYFYPEAPRFDYFVFDLFHELKPLPPLERNELLEKYGLKHVRLLGVIDKNDVEMFKQIVAELDREGREGVVAKDPEYRVPPLKYTTSAVNIGDVRYGMRFFMEEGRSFLFSRLLRELFRAYEEGFGDAQLEKLALEFGRAATEPALESIRKVAMGDMLYEEFELVFADEVELEEFTSYMAELGVDIVVVSTSREDEGLRARMRKIKDTWIQLRKVLDTGLSPVD

SEQ ID NO: 3 - protein, 390 aa, artificial sequence
  R281 mutant of HyperLigase
  misc_feature (281)..(281): Xaa can be any amino acid except Arg
MTWIKNPEPWMVNLVAEKLGLDVERVETLARHGTIRFRGYRDVVYALLRREIAGHPEGTVVLLERNGARLVPGYPPIQRMVLPTIALPRHFIDKVVVEEAMNGYNVRLVMFHRKLLAVTRGGFICPYTTARLERLIGGRVRELFREIDPETYTIAGEVVGLENPYTRYFYPEAPRFDYFVFDLFHELKPLPPLERNELLEKYGLKHVRLLGVIDKNDVEMFKQIVAELDREGREGVVAKDPEYRVPPLKYTTSAVNIGDVRYGMRFFMEEGRSFLFSRLLXELFRAYEEGFGDAQLEKLALEFGRAATEPALESIRKVAMGDMLYEEFELVFADEVELEEFTSYMAELGVDIVVVSTSREDEGLRARMRKIKDTWIQLRKVLDTGLSPVD

SEQ ID NO: 4 - protein, 390 aa, artificial sequence
  K370 mutant of Hyperligase
  misc_feature (370)..(370): Xaa can be any amino acid except Lys
MTWIKNPEPWMVNLVAEKLGLDVERVETLARHGTIRFRGYRDVVYALLRREIAGHPEGTVVLLERNGARLVPGYPPIQRMVLPTIALPRHFIDKVVVEEAMNGYNVRLVMFHRKLLAVTRGGFICPYTTARLERLIGGRVRELFREIDPETYTIAGEVVGLENPYTRYFYPEAPRFDYFVFDLFHELKPLPPLERNELLEKYGLKHVRLLGVIDKNDVEMFKQIVAELDREGREGVVAKDPEYRVPPLKYTTSAVNIGDVRYGMRFFMEEGRSFLFSRLLRELFRAYEEGFGDAQLEKLALEFGRAATEPALESIRKVAMGDMLYEEFELVFADEVELEEFTSYMAELGVDIVVVSTSREDEGLRARMRXIKDTWIQLRKVLDTGLSPVD

SEQ ID NO: 5 - protein, 390 aa, artificial sequence
  K372 mutant of HyperLigase
  misc_feature (372)..(372): Xaa can be any amino acid except Lys
MTWIKNPEPWMVNLVAEKLGLDVERVETLARHGTIRFRGYRDVVYALLRREIAGHPEGTVVLLERNGARLVPGYPPIQRMVLPTIALPRHFIDKVVVEEAMNGYNVRLVMFHRKLLAVTRGGFICPYTTARLERLIGGRVRELFREIDPETYTIAGEVVGLENPYTRYFYPEAPRFDYFVFDLFHELKPLPPLERNELLEKYGLKHVRLLGVIDKNDVEMFKQIVAELDREGREGVVAKDPEYRVPPLKYTTSAVNIGDVRYGMRFFMEEGRSFLFSRLLRELFRAYEEGFGDAQLEKLALEFGRAATEPALESIRKVAMGDMLYEEFELVFADEVELEEFTSYMAELGVDIVVVSTSREDEGLRARMRKIXDTWIQLRKVLDTGLSPVD

SEQ ID NO: 6 - protein, 390 aa, artificial sequence
  combined K370 and K372 mutant of HyperLigase
  misc_feature (370)..(370): Xaa can be any amino acid except Lys
  misc_feature (372)..(372): Xaa can be any amino acid except Lys
MTWIKNPEPWMVNLVAEKLGLDVERVETLARHGTIRFRGYRDVVYALLRREIAGHPEGTVVLLERNGARLVPGYPPIQRMVLPTIALPRHFIDKVVVEEAMNGYNVRLVMFHRKLLAVTRGGFICPYTTARLERLIGGRVRELFREIDPETYTIAGEVVGLENPYTRYFYPEAPRFDYFVFDLFHELKPLPPLERNELLEKYGLKHVRLLGVIDKNDVEMFKQIVAELDREGREGVVAKDPEYRVPPLKYTTSAVNIGDVRYGMRFFMEEGRSFLFSRLLRELFRAYEEGFGDAQLEKLALEFGRAATEPALESIRKVAMGDMLYEEFELVFADEVELEEFTSYMAELGVDIVVVSTSREDEGLRARMRXIXDTWIQLRKVLDTGLSPVD

SEQ ID NO: 7 - protein, 390 aa, artificial sequence
  four-site mutant of Hyperligase
  misc_feature (79)..(79): Xaa can be any amino acid except Arg
  misc_feature (281)..(281): Xaa can be any amino acid except Arg
  misc_feature (370)..(370): Xaa can be any amino acid except Lys
  misc_feature (372)..(372): Xaa can be any amino acid except Lys
MTWIKNPEPWMVNLVAEKLGLDVERVETLARHGTIRFRGYRDVVYALLRREIAGHPEGTVVLLERNGARLVPGYPPIQXMVLPTIALPRHFIDKVVVEEAMNGYNVRLVMFHRKLLAVTRGGFICPYTTARLERLIGGRVRELFREIDPETYTIAGEVVGLENPYTRYFYPEAPRFDYFVFDLFHELKPLPPLERNELLEKYGLKHVRLLGVIDKNDVEMFKQIVAELDREGREGVVAKDPEYRVPPLKYTTSAVNIGDVRYGMRFFMEEGRSFLFSRLLXELFRAYEEGFGDAQLEKLALEFGRAATEPALESIRKVAMGDMLYEEFELVFADEVELEEFTSYMAELGVDIVVVSTSREDEGLRARMRXIXDTWIQLRKVLDTGLSPVD